European Patent Application EP 4 425 500 A2, published September 4, 2024. Title: ALIGNMENT AND VARIANT SEQUENCING ANALYSIS PIPELINE. Applicant: QUEST DIAGNOSTICS INVESTMENTS INCORPORATED. The sequence listing filed with the application follows.

SEQUENCE LISTING (6 sequences)

SEQ ID NO: 1 - DNA, 11 bp, Homo sapiens
  source 1..11: mol_type = unassigned DNA
gaagatactag

SEQ ID NO: 2 - DNA, 41 bp, Homo sapiens
  source 1..41: mol_type = unassigned DNA
tgattcagactccccatcatgtgagtcatcagaacctaaca

SEQ ID NO: 3 - DNA, 93 bp, Homo sapiens
  source 1..93: mol_type = unassigned DNA
agcattcagatctacctttttttctgtgctgggagtccgcctatcattacatgtttccttacttccagcccatctgttatgttggctccttgc

SEQ ID NO: 4 - protein, 31 aa, Homo sapiens
ANLDVKKETSPTRRDNCTEKSGAWRNHQSRA

SEQ ID NO: 5 - DNA, 66 bp, Homo sapiens
  source 1..66: mol_type = unassigned DNA
aaaatgactctaggtcaagatttaaaatcggacatctccttgaatatagataaaataccagaaaaa

SEQ ID NO: 6 - protein, 22 aa, Homo sapiens
KMTLGQDLKSDISLNIDKIPEK